European Patent Application EP 4 372 088 A1, published May 22, 2024. Title: Anti-EGFRviii antibody, polypeptide, cell expressing the polypeptide, pharmaceutical composition including the cell, method of producing the cell, and polynucleotide or vector including base sequence encoding the polypeptide. Applicant: Noile-Immune Biotech Inc. The sequence listing filed with the application follows.

SEQUENCE LISTING (54 sequences)

SEQ ID NO: 1 - protein, 116 aa, synthetic construct
  REGION 1..116: note = VH region of anti-EGFRviii antibody for VL15VH 1B10-1A12E
QVTLKESGPGILQPSQTLSLTCSFSGFSLSTSGMGVSWIRQPSGKGLEWLAHIFWDDDKRYNPSLKSRLTISKDTSTNQVFLKITSVDTADTATYYCARNYGFDVWGAGTTVTVSS

SEQ ID NO: 2 - protein, 112 aa, synthetic construct
  REGION 1..112: note = VL region of antiEGFRviii antibody for 1B10-1A12
DVVMTQTPLSLPVSLEDQASISCRSSQSLVHSNGKTYLQWYLQKPGQSPKLLIYSVSNRFSGVPDRFSGSGSGRDFTLKISRVEAEDLGVYFCSQSTHVPWTFGGGTKLEIK

SEQ ID NO: 3 - protein, 112 aa, synthetic construct
  REGION 1..112: note = VL region of antiEGFRviii antibody for 1B10-1A12
DVVMTQTPLSLPVSLEDQASISCRSSQSLVHSSGKTYLQWYLQKPGQSPKLLIYSVSNRFSGVPDRFSGSGSGRDFTLKISRVEAEDLGVYFCSQSTHVPWTFGGGTKLEIK

SEQ ID NO: 4 - protein, 116 aa, synthetic construct
  REGION 1..116: note = VH region of antiEGFRviii antibody for 1B10-1A12
QVTLKESGPALVKPTQTLTLTCTFSGFSLSTSGMGVSWIRQPPGKALEWLAHIFWDDDKRYNPSLKSRLTISKDTSKNQVVLTMTNMDPVDTATYYCARNYGFDVWGQGTLVTVSS

SEQ ID NO: 5 - protein, 112 aa, synthetic construct
  REGION 1..112: note = VL region of antiEGFRviii antibody for 1B10-1A12
DIVMTQSPLSLPVTPGEPASISCRSSQSLVHSSGKTYLQWYLQKPGQSPQLLIYSVSNRFSGVPDRFSGSGSGRDFTLKISRVEAEDVGVYYCSQSTHVPWTFGGGTKVEIK

SEQ ID NO: 6 - protein, 112 aa, synthetic construct
  REGION 1..112: note = VL region of antiEGFRviii antibody for 1B10-1A12
DIVMTQSPLSLPVTPGEPASISCRSSQSLVHSSGKTYLQWYLQKPGQSPQLLIYSVSNRFSGVPDRFSGSGSGRDFTLKISRVEAEDVGVYYCSQSTHVPWTFGGGTKLEIK

SEQ ID NO: 7 - DNA, 336 bp, synthetic construct
  misc_feature 1..336: note = VL region of antiEGFRviii antibody for 1B10-1A12
  source 1..336: mol_type = other DNA
gatatcgtgatgacccagagccctctgtccctccccgtgacacccggcgagcccgcctccatcagctgtagatcctcccagtccctcgtgcactcctccggcaagacctacctccaatggtacctccagaagcccggccagagcccccagctcctcatctacagcgtgtccaacagattcagcggagtccccgacagattcagcggaagcggcagcggaagagactttacactgaagatctctagagtggaagccgaggatgtgggcgtctactactgtagccaaagcacccacgtgccttggacattcggaggaggcaccaaactcgagatcaag

SEQ ID NO: 8 - DNA, 348 bp, synthetic construct
  misc_feature 1..348: note = VH region of antiEGFRviii antibody for 1B10-1A12
  source 1..348: mol_type = other DNA
caagtgacactgaaggaatccggacccgctctggtgaagcctacccagaccctcacactgacatgcacattcagcggcttttctctgtccacatccggcatgggcgtcagctggattagacagcctcccggcaaagctctggagtggctcgcccacatcttctgggacgacgacaagaggtacaacccctctctgaagtctagactgaccatcagcaaggacaccagcaagaaccaagtggtcctcaccatgaccaacatggatcccgtggacaccgccacctattactgtgctaggaactacggcttcgacgtctggggccaaggcacactggtgacagtctccagc

SEQ ID NO: 9 - DNA, 729 bp, synthetic construct
  misc_feature 1..729: note = anti-EGFRviii scFv VL15VH
  source 1..729: mol_type = other DNA
gatatcgtgatgacccagagccctctgtccctccccgtgacacccggcgagcccgcctccatcagctgtagatcctcccagtccctcgtgcactcctccggcaagacctacctccaatggtacctccagaagcccggccagagcccccagctcctcatctacagcgtgtccaacagattcagcggagtccccgacagattcagcggaagcggcagcggaagagactttacactgaagatctctagagtggaagccgaggatgtgggcgtctactactgtagccaaagcacccacgtgccttggacattcggaggaggcaccaaactcgagatcaagggcggcggagggtcaggcggtggcgggtctggcggtggaggatcccaagtgacactgaaggaatccggacccgctctggtgaagcctacccagaccctcacactgacatgcacattcagcggcttttctctgtccacatccggcatgggcgtcagctggattagacagcctcccggcaaagctctggagtggctcgcccacatcttctgggacgacgacaagaggtacaacccctctctgaagtctagactgaccatcagcaaggacaccagcaagaaccaagtggtcctcaccatgaccaacatggatcccgtggacaccgccacctattactgtgctaggaactacggcttcgacgtctggggccaaggcacactggtgacagtctccagc

SEQ ID NO: 10 - DNA, 759 bp, synthetic construct
  misc_feature 1..759: note = anti-EGFRviiiscFv for VL25VH
  source 1..759: mol_type = other DNA
gatatcgtgatgacccagagccctctgtccctccccgtgacacccggcgagcccgcctccatcagctgtagatcctcccagtccctcgtgcactcctccggcaagacctacctccaatggtacctccagaagcccggccagagcccccagctcctcatctacagcgtgtccaacagattcagcggagtccccgacagattcagcggaagcggcagcggaagagactttacactgaagatctctagagtggaagccgaggatgtgggcgtctactactgtagccaaagcacccacgtgccttggacattcggaggaggcaccaaactcgagatcaagagcagcgccgatgacgctaaaaaggacgccgccaaaaaggacgacgctaagaaagacgacgccaagaaggatggacaagtgacactgaaggaatccggacccgctctggtgaagcctacccagaccctcacactgacatgcacattcagcggcttttctctgtccacatccggcatgggcgtcagctggattagacagcctcccggcaaagctctggagtggctcgcccacatcttctgggacgacgacaagaggtacaacccctctctgaagtctagactgaccatcagcaaggacaccagcaagaaccaagtggtcctcaccatgaccaacatggatcccgtggacaccgccacctattactgtgctaggaactacggcttcgacgtctggggccaaggcacactggtgacagtctccagc

SEQ ID NO: 11 - DNA, 9272 bp, synthetic construct
  misc_feature 1..9272: note = anti EGFRviii CAR for 1B10-1A12
  source 1..9272: mol_type = other DNA
ccatggactggacatggaggattctgtttctggtggctgctgccaccggcgctcattccgatatcgtgatgacccagagccctctgtccctccccgtgacacccggcgagcccgcctccatcagctgtagatcctcccagtccctcgtgcactcctccggcaagacctacctccaatggtacctccagaagcccggccagagcccccagctcctcatctacagcgtgtccaacagattcagcggagtccccgacagattcagcggaagcggcagcggaagagactttacactgaagatctctagagtggaagccgaggatgtgggcgtctactactgtagccaaagcacccacgtgccttggacattcggaggaggcaccaaactcgagatcaagagcagcgccgatgacgctaaaaaggacgccgccaaaaaggacgacgctaagaaagacgacgccaagaaggatggacaagtgacactgaaggaatccggacccgctctggtgaagcctacccagaccctcacactgacatgcacattcagcggcttttctctgtccacatccggcatgggcgtcagctggattagacagcctcccggcaaagctctggagtggctcgcccacatcttctgggacgacgacaagaggtacaacccctctctgaagtctagactgaccatcagcaaggacaccagcaagaaccaagtggtcctcaccatgaccaacatggatcccgtggacaccgccacctattactgtgctaggaactacggcttcgacgtctggggccaaggcacactggtgacagtctccagcgctgctgctaccaccacacccgctcctaggcctcctacacccgcccctacaatcgctagccagcctctgagcctcagacccgaggcttgcagacccgctgctggcggagctgtccacaccagaggactggacttcgcttgcgatatctacatttgggctcctctggccggaacatgcggagtgctgctgctgagcctcgtgattacactgagattcagcgtggtgaagaggggaagaaagaagctgctgtatattttcaagcagcccttcatgaggcccgtgcaaacaacccaagaggaagatggctgcagctgtagattccccgaagaggaggagggcggctgtgaactgagggtcaaattctctagaagcgctgatgcccccgcctaccaacaaggccagaaccagctgtacaacgaactgaacctcggaaggagagaagagtacgacgtgctggacaaaagaaggggaagagaccccgagatgggcggcaagcccagaagaaagaacccccaagagggcctctacaacgagctgcagaaggacaaaatggctgaggcctactccgagattggcatgaagggcgaaagaaggaggggcaaaggccacgatggactgtaccaaggcctcagcaccgccaccaaggacacctatgatgctctgcacatgcaagctctgccccccagagaattcggaagcggagtgaaacagactttgaattttgaccttctcaagttggcgggagacgtggagtccaaccctggaccatgcatgttccatgtgagcttcaggtacatcttcggactgcctcctctcatcctggtcctcctccccgtggccagctccgactgtgacatcgaaggaaaggatggcaagcagtacgaaagcgtgctgatggtgagcatcgatcagctcctggattccatgaaggaaatcggctccaactgcctcaacaatgagttcaacttttttaagaggcatatctgcgacgccaacaaggagggcatgtttctgttcagggccgccaggaagctgagacagttcctcaagatgaatagcaccggcgacttcgacctccatctgctgaaggtgtccgagggaaccaccatcctgctgaactgcaccggccaagtgaagggaagaaaacctgctgccctgggcgaggctcagcctaccaagagcctcgaggagaacaaaagcctgaaggagcagaagaagctgaacgacctgtgcttcctcaagaggctcctgcaggagattaagacctgttggaacaagatcctgatgggcacaaaggagcacggatccggcgtgaagcagaccctgaactttgacctgctcaaactggccggcgacgtcgagtccaatcctggacctatggctctgctgctcgccctgagcctgctcgtcctctggacctcccctgctcctaccctgagcggcaccaatgacgctgaagactgctgcctgtccgtgacccagaagcctatccccggatatatcgtgaggaattttcattacctcctgatcaaggacggctgtagagtgcccgccgtcgtgttcacaacactcagaggcaggcagctgtgtgctccccccgaccagccttgggtggagagaatcattcagagactgcaaaggacctccgctaagatgaagaggaggtccagcggcagcggagtgaagcagacactgaatttcgacctgctcaagctggccggcgatgtggagagcaaccctggacctatggcttcctaccccggacatcagcacgcttccgccttcgaccaggccgctagaagcagaggacactccaatagaaggacagccctgaggcctaggagacagcaggaggccaccgaggtgaggcccgagcagaaaatgcccaccctgctgagagtgtatattgatggaccccacggcatgggaaaaaccaccacaacccagctgctggtggctctgggaagcagggatgatattgtgtacgtccccgaacctatgacatattggagggtcctcggcgcctccgagaccatcgccaacatttacaccacccagcacaggctggatcagggagagatctccgccggcgatgctgccgtggtgatgaccagcgcccagatcactatgggtatgccttatgccgtgaccgacgctgtgctggctcctcacattggcggcgaagccggatcctcccatgctccccctcctgccctcacactgatctttgacagacatcctatcgccgctctgctgtgctaccccgccgctaggtacctgatgggcagcatgacccctcaggccgtgctggcttttgtggccctcattccccccacactgcctggcacaaatatcgtgctcggcgccctgcctgaggacaggcacatcgataggctggctaagagacagagacccggagagaggctggatctcgctatgctggccgccatcaggagggtgtacggcctgctggccaacaccgtgagatatctccagtgtggcggatcctggagggaagactggggccaactgagcggcacagctgtgcctcctcaaggcgctgagccccagagcaacgctggacccagacctcacatcggcgataccctgttcaccctgtttagagcccctgagctcctggcccctaacggcgacctgtacaatgtgttcgcttgggccctggatgtgctcgccaagagactcaggagcatgcacgtcttcattctggactacgaccagtcccccgctggctgcagagatgccctgctccagctgacctccggcatggtgcagacccacgtgaccacccctggaagcatccccacaatctgcgacctggccaggacctttgccagagaaatgggagaagccaactgagtcgacaaaggccaaaaaggccaacgtacgaaggatccgataaaataaaagattttatttagtctccagaaaaaggggggaatgaaagaccccacctgtaggtttggcaagctagcttaagtaacgccattttgcaaggcatggaaaatacataactgagaatagagaagttcagatcaaggttaggaacagagagacagcagaatatgggccaaacaggatatctgtggtaagcagttcctgccccggctcagggccaagaacagatggtccccagatgcggtcccgccctcagcagtttctagagaaccatcagatgtttccagggtgccccaaggacctgaaatgaccctgtgccttatttgaactaaccaatcagttcgcttctcgcttctgttcgcgcgcttctgctccccgagctcaataaaagagcccacaacccctcactcggcgcgccagtcctccgatagactgcgtcgcccgggtacccgtgtatccaataaaccctcttgcagttgcatccgacttgtggtctcgctgttccttgggagggtctcctctgagtgattgactacccgtcagcgggggtctttcatgggtaacagtttcttgaagttggagaacaacattctgagggtaggagtcgaatattaagtaatcctgactcaattagccactgttttgaatccacatactccaatactcctgaaatccatcgatggagttcattatggacagcgcagaaagagctggggagaattgtgaaattgttatccgctcacaattccacacaacatacgagccggaagcataaagtgtaaagcctggggtgcctaatgagtgagctaactcacattaattgcgttgcgctcactgcccgctttccagtcgggaaacctgtcgtgccagctgcattaatgaatcggccaacgcgcggggagaggcggtttgcgtattgggcgctcttccgcttcctcgctcactgactcgctgcgctcggtcgttcggctgcggcgagcggtatcagctcactcaaaggcggtaatacggttatccacagaatcaggggataacgcaggaaagaacatgtgagcaaaaggccagcaaaaggccaggaaccgtaaaaaggccgcgttgctggcgtttttccataggctccgcccccctgacgagcatcacaaaaatcgacgctcaagtcagaggtggcgaaacccgacaggactataaagataccaggcgtttccccctggaagctccctcgtgcgctctcctgttccgaccctgccgcttaccggatacctgtccgcctttctcccttcgggaagcgtggcgctttctcatagctcacgctgtaggtatctcagttcggtgtaggtcgttcgctccaagctgggctgtgtgcacgaaccccccgttcagcccgaccgctgcgccttatccggtaactatcgtcttgagtccaacccggtaagacacgacttatcgccactggcagcagccactggtaacaggattagcagagcgaggtatgtaggcggtgctacagagttcttgaagtggtggcctaactacggctacactagaagaacagtatttggtatctgcgctctgctgaagccagttaccttcggaaaaagagttggtagctcttgatccggcaaacaaaccaccgctggtagcggtggtttttttgtttgcaagcagcagattacgcgcagaaaaaaaggatctcaagaagatcctttgatcttttctacggggtctgacgctcagtggaacgaaaactcacgttaagggattttggtcatgagattatcaaaaaggatcttcacctagatccttttaaattaaaaatgaagttttaaatcaatctaaagtatatatgagtaaacttggtctgacagttaccaatgcttaatcagtgaggcacctatctcagcgatctgtctatttcgttcatccatagttgcctgactccccgtcgtgtagataactacgatacgggagggcttaccatctggccccagtgctgcaatgataccgcgagacccacgctcaccggctccagatttatcagcaataaaccagccagccggaagggccgagcgcagaagtggtcctgcaactttatccgcctccatccagtctattaattgttgccgggaagctagagtaagtagttcgccagttaatagtttgcgcaacgttgttgccattgctacaggcatcgtggtgtcacgctcgtcgtttggtatggcttcattcagctccggttcccaacgatcaaggcgagttacatgatcccccatgttgtgcaaaaaagcggttagctccttcggtcctccgatcgttgtcagaagtaagttggccgcagtgttatcactcatggttatggcagcactgcataattctcttactgtcatgccatccgtaagatgcttttctgtgactggtgagtactcaaccaagtcattctgagaatagtgtatgcggcgaccgagttgctcttgcccggcgtcaatacgggataataccgcgccacatagcagaactttaaaagtgctcatcattggaaaacgttcttcggggcgaaaactctcaaggatcttaccgctgttgagatccagttcgatgtaacccactcgtgcacccaactgatcttcagcatcttttactttcaccagcgtttctgggtgagcaaaaacaggaaggcaaaatgccgcaaaaaagggaataagggcgacacggaaatgttgaatactcatactcttcctttttcaatattattgaagcatttatcagggttattgtctcatgagcggatacatatttgaatgtatttagaaaaataaacaaataggggttccgcgcacatttccccgaaaagtgccacctgacgtctaagaaaccattattatcatgacattaacctataaaaataggcgtatcacgaggccctttcgtctcgcgcgtttcggtgatgacggtgaaaacctctgacacatgcagctcccggagacggtcacagcttgtctgtaagcggatgccgggagcagacaagcccgtcagggcgcgtcagcgggtgttggcgggtgtcggggctggcttaactatgcggcatcagagcagattgtactgagagtgcaccatatgcggtgtgaaataccgcacagatgcgtaaggagaaaataccgcatcaggcgccattcgccattcaggctgcgcaactgttgggaagggcgatcggtgcgggcctcttcgctattacgccagctggcgaaagggggatgtgctgcaaggcgattaagttgggtaacgccagggttttcccagtcacgacgttgtaaaacgacggccagtgccacgctctcccttatgcgactcctgcattaggaagcagcccagtagtaggttgaggccgttgagcaccgccgccgcaaggaatggtgcatgcaaggagatggcgcccaacagtcccccggccacggggcctgccaccatacccacgccgaaacaagcgctcatgagcccgaagtggcgagcccgatcttccccatcggtgatgtcggcgatataggcgccagcaaccgcacctgtggcgccggtgatgccggccacgatgcgtccggcgtagaggcgatttaaagacaggatatcagtggtccaggctctagttttgactcaacaatatcaccagctgaagcctatagagtacgagccatagataaaataaaagattttatttagtctccagaaaaaggggggaatgaaagaccccacctgtaggtttggcaagctagcttaagtaacgccattttgcaaggcatggaaaatacataactgagaatagagaagttcagatcaaggttaggaacagagagacagcagaatatgggccaaacaggatatctgtggtaagcagttcctgccccggctcagggccaagaacagatggtccccagatgcggtcccgccctcagcagtttctagagaaccatcagatgtttccagggtgccccaaggacctgaaaatgaccctgtgccttatttgaactaaccaatcagttcgcttctcgcttctgttcgcgcgcttctgctccccgagctcaataaaagagcccacaacccctcactcggcgcgccagtcctccgatagactgcgtcgcccgggtacccgtattcccaataaagcctcttgctgtttgcatccgaatcgtggactcgctgatccttgggagggtctcctcagattgattgactgcccacctcgggggtctttcatttggaggttccaccgagatttggagacccctgcctagggaccaccgacccccccgccgggaggtaagctggccagcggtcgtttcgtgtctgtctctgtctttgtgcgtgtttgtgccggcatctaatgtttgcgcctgcgtctgtactagttagctaactagctctgtatctggcggacccgtggtggaactgacgagttcggaacacccggccgcaaccctgggagacgtcccagggacttcgggggccgtttttgtggcccgacctgagtccaaaaatcccgatcgttttggactctttggtgcaccccccttagaggagggatatgtggttctggtaggagacgagaacctaaaacagttcccgcctccgtctgaatttttgctttcggtttgggaccgaagccgcgccgcgcgtcttgtctgctgcagcatcgttctgtgttgtctctgtctgactgtgtttctgtatttgtctgagaatatgggcccgggctagcctgttaccactcccttaagtttgaccttaggtcactggaaagatgtcgagcggatcgctcacaaccagtcggtagatgtcaagaagagacgttgggttaccttctgctctgcagaatggccaacctttaacgtcggatggccgcgagacggcacctttaaccgagacctcatcacccaggttaagatcaaggtcttttcacctggcccgcatggacacccagaccaggtcccctacatcgtgacctgggaagccttggcttttgacccccctccctgggtcaagccctttgtacaccctaagcctccgcctcctcttcctccatccgccccgtctctcccccttgaacctcctcgttcgaccccgcctcgatcctccctttatccagccctcactccttctctaggcgcccccatatggccatatgagatcttatatggggcacccccgccccttgtaaacttccctgaccctgacatgacaagagttactaacagcccctctctccaagctcacttacaggctctctacttagtccagcacgaagtctggagacctctggcggcagcctaccaagaacaactggaccgaccggtggtacctcacccttaccgagtcggcgacacagtgtgggtccgccgacaccagactaagaacctagaacctcgctggaaaggaccttacacagtcctgctgaccacccccaccgccctcaaagtagacggcatcgcagcttggatacacgccgcccacgtgaaggctgccgaccccgggggtggaccatcctctagaccg

SEQ ID NO: 12 - protein, 243 aa, synthetic construct
  REGION 1..243: note = anti-EGFRviii scFvVH-15-VL
QVTLKESGPALVKPTQTLTLTCTFSGFSLSTSGMGVSWIRQPPGKALEWLAHIFWDDDKRYNPSLKSRLTISKDTSKNQVVLTMTNMDPVDTATYYCARNYGFDVWGQGTLVTVSSGGGGSGGGGSGGGGSDIVMTQSPLSLPVTPGEPASISCRSSQSLVHSSGKTYLQWYLQKPGQSPQLLIYSVSNRFSGVPDRFSGSGSGRDFTLKISRVEAEDVGVYYCSQSTHVPWTFGGGTKLEIK

SEQ ID NO: 13 - protein, 243 aa, synthetic construct
  REGION 1..243: note = anti-EGFRviii scFv VL-15-VHFS#020
DVVMTQTPLSLPVSLEDQASISCRSSQSLVHSSGKTYLQWYLQKPGQSPKLLIYSVSNRFSGVPDRFSGSGSGRDFTLKISRVEAEDLGVYFCSQSTHVPWTFGGGTKLEIKGGGGSGGGGSGGGGSQVTLKESGPGILQPSQTLSLTCSFSGFSLSTSGMGVSWIRQPSGKGLEWLAHIFWDDDKRYNPSLKSRLTISKDTSTNQVFLKITSVDTADTATYYCARNYGFDVWGAGTTVTVSS

SEQ ID NO: 14 - protein, 243 aa, synthetic construct
  REGION 1..243: note = nti-EGFRviii scFv VH-15-VLFS#021
QVTLKESGPGILQPSQTLSLTCSFSGFSLSTSGMGVSWIRQPSGKGLEWLAHIFWDDDKRYNPSLKSRLTISKDTSTNQVFLKITSVDTADTATYYCARNYGFDVWGAGTTVTVSSGGGGSGGGGSGGGGSDVVMTQTPLSLPVSLEDQASISCRSSQSLVHSSGKTYLQWYLQKPGQSPKLLIYSVSNRFSGVPDRFSGSGSGRDFTLKISRVEAEDLGVYFCSQSTHVPWTFGGGTKLEIK

SEQ ID NO: 15 - protein, 253 aa, synthetic construct
  REGION 1..253: note = anti-EGFRviii scFv VL-15-VHFS#022
DVVMTQTPLSLPVSLEDQASISCRSSQSLVHSSGKTYLQWYLQKPGQSPKLLIYSVSNRFSGVPDRFSGSGSGRDFTLKISRVEAEDLGVYFCSQSTHVPWTFGGGTKLEIKSSADDAKKDAAKKDDAKKDDAKKDGQVTLKESGPGILQPSQTLSLTCSFSGFSLSTSGMGVSWIRQPSGKGLEWLAHIFWDDDKRYNPSLKSRLTISKDTSTNQVFLKITSVDTADTATYYCARNYGFDVWGAGTTVTVSS

SEQ ID NO: 16 - protein, 253 aa, synthetic construct
  REGION 1..253: note = anti-EGFRviii scFv VH-25-VLFS#023
QVTLKESGPGILQPSQTLSLTCSFSGFSLSTSGMGVSWIRQPSGKGLEWLAHIFWDDDKRYNPSLKSRLTISKDTSTNQVFLKITSVDTADTATYYCARNYGFDVWGAGTTVTVSSSSADDAKKDAAKKDDAKKDDAKKDGDVVMTQTPLSLPVSLEDQASISCRSSQSLVHSSGKTYLQWYLQKPGQSPKLLIYSVSNRFSGVPDRFSGSGSGRDFTLKISRVEAEDLGVYFCSQSTHVPWTFGGGTKLEIK

SEQ ID NO: 17 - protein, 243 aa, synthetic construct
  REGION 1..243: note = anti-EGFRviii scFv VL-15-VHEhumanized
DIVMTQSPLSLPVTPGEPASISCRSSQSLVHSSGKTYLQWYLQKPGQSPQLLIYSVSNRFSGVPDRFSGSGSGRDFTLKISRVEAEDVGVYYCSQSTHVPWTFGGGTKLEIKGGGGSGGGGSGGGGSQVTLKESGPALVKPTQTLTLTCTFSGFSLSTSGMGVSWIRQPPGKALEWLAHIFWDDDKRYNPSLKSRLTISKDTSKNQVVLTMTNMDPVDTATYYCARNYGFDVWGQGTLVTVSS

SEQ ID NO: 18 - protein, 253 aa, synthetic construct
  REGION 1..253: note = anti-EGFRviii scFv VL-25-VHEhumanized
DIVMTQSPLSLPVTPGEPASISCRSSQSLVHSSGKTYLQWYLQKPGQSPQLLIYSVSNRFSGVPDRFSGSGSGRDFTLKISRVEAEDVGVYYCSQSTHVPWTFGGGTKLEIKSSADDAKKDAAKKDDAKKDDAKKDGQVTLKESGPALVKPTQTLTLTCTFSGFSLSTSGMGVSWIRQPPGKALEWLAHIFWDDDKRYNPSLKSRLTISKDTSKNQVVLTMTNMDPVDTATYYCARNYGFDVWGQGTLVTVSS

SEQ ID NO: 19 - protein, 22 aa, synthetic construct
  REGION 1..22: note = CD8a transmembrane region short
IYIWAPLAGTCGVLLLSLVITL

SEQ ID NO: 20 - protein, 29 aa, synthetic construct
  REGION 1..29: note = CD8a transmembrane region long
IYIWAPLAGTCGVLLLSLVITLYCNHRNR

SEQ ID NO: 21 - protein, 45 aa, synthetic construct
  REGION 1..45: note = CD8a hinge region short
TTTPAPRPPTPAPTIASQPLSLRPEACRPAAGGAVHTRGLDFACD

SEQ ID NO: 22 - protein, 55 aa, synthetic construct
  REGION 1..55: note = CD8a hinge region long
FVPVFLPAKPTTTPAPRPPTPAPTIASQPLSLRPEACRPAAGGAVHTRGLDFACD

SEQ ID NO: 23 - protein, 19 aa, synthetic construct
  REGION 1..19: note = signal sequence IgG SS long
MDWTWRILFLVAAATGAHS

SEQ ID NO: 24 - protein, 21 aa, synthetic construct
  REGION 1..21: note = signal sequence CD8 SS long
MALPVTALLLPLALLLHAARP

SEQ ID NO: 25 - protein, 113 aa, Homo sapiens
LRVKFSRSADAPAYQQGQNQLYNELNLGRREEYDVLDKRRGRDPEMGGKPRRKNPQEGLYNELQKDKMAEAYSEIGMKGERRRGKGHDGLYQGLSTATKDTYDALHMQALPPR

SEQ ID NO: 26 - protein, 41 aa, synthetic construct
  REGION 1..41: note = CD28 T-cell signal transduction region
RSKRSRLLHSDYMNMTPRRPGPTRKHYQPYAPPRDFAAYRS

SEQ ID NO: 27 - protein, 46 aa, synthetic construct
  REGION 1..46: note = 4-1BB signal transduction region
RFSVVKRGRKKLLYIFKQPFMRPVQTTQEEDGCSCRFPEEEEGGCE

SEQ ID NO: 28 - protein, 177 aa, Homo sapiens
MFHVSFRYIFGLPPLILVLLPVASSDCDIEGKDGKQYESVLMVSIDQLLDSMKEIGSNCLNNEFNFFKRHICDANKEGMFLFRAARKLRQFLKMNSTGDFDLHLLKVSEGTTILLNCTGQVKGRKPAALGEAQPTKSLEENKSLKEQKKLNDLCFLKRLLQEIKTCWNKILMGTKEH

SEQ ID NO: 29 - protein, 98 aa, Homo sapiens
MALLLALSLLVLWTSPAPTLSGTNDAEDCCLSVTQKPIPGYIVRNFHYLLIKDGCRVPAVVFTTLRGRQLCAPPDQPWVERIIQRLQRTSAKMKRRSS

SEQ ID NO: 30 - protein, 67 aa, synthetic construct
  REGION 1..67: note = CD8a hinge and transmembrane region short
TTTPAPRPPTPAPTIASQPLSLRPEACRPAAGGAVHTRGLDFACDIYIWAPLAGTCGVLLLSLVITL

SEQ ID NO: 31 - protein, 12 aa, synthetic construct
  REGION 1..12: note = heavy chain CDR1 of 1B10-1A12
GFSLSTSGMGVS

SEQ ID NO: 32 - protein, 14 aa, synthetic construct
  REGION 1..14: note = heavy chain CDR2 of 1B10-1A12
HIFWDDDKRYNPSL

SEQ ID NO: 33 - protein, 6 aa, synthetic construct
  REGION 1..6: note = heavy chain CDR3 of 1B10-1A12
NYGFDV

SEQ ID NO: 34 - protein, 16 aa, synthetic construct
  REGION 1..16: note = light chain CDR1 (SG) of 1B10-1A12
RSSQSLVHSSGKTYLQ

SEQ ID NO: 35 - protein, 7 aa, synthetic construct
  REGION 1..7: note = light chain CDR2 of 1B10-1A12
SVSNRFS

SEQ ID NO: 36 - protein, 9 aa, synthetic construct
  REGION 1..9: note = light chain CDR3 of 1B10-1A12
SQSTHVPWT

SEQ ID NO: 37 - protein, 16 aa, synthetic construct
  REGION 1..16: note = light chain CDR1 (NG) of 1B10-1A12
RSSQSLVHSNGKTYLQ

SEQ ID NO: 38 - protein, 253 aa, synthetic construct
  REGION 1..253: note = anti-EGFRviii scFv VH-25-VL (humanized)
QVTLKESGPALVKPTQTLTLTCTFSGFSLSTSGMGVSWIRQPPGKALEWLAHIFWDDDKRYNPSLKSRLTISKDTSKNQVVLTMTNMDPVDTATYYCARNYGFDVWGQGTLVTVSSSSADDAKKDAAKKDDAKKDDAKKDGDIVMTQSPLSLPVTPGEPASISCRSSQSLVHSSGKTYLQWYLQKPGQSPQLLIYSVSNRFSGVPDRFSGSGSGRDFTLKISRVEAEDVGVYYCSQSTHVPWTFGGGTKLEIK

SEQ ID NO: 39 - protein, 8 aa, synthetic construct
  REGION 1..8: note = 2A peptide cleavage region
  SITE 2: note = misc_feature - Xaa can be any naturally occurring amino acid
  SITE 4: note = misc_feature - Xaa can be any naturally occurring amino acid
DXEXNPGP

SEQ ID NO: 40 - protein, 25 aa, synthetic construct
  REGION 1..25: note = F2A
GSGVKQTLNFDLLKLAGDVESNPGP

SEQ ID NO: 41 - protein, 15 aa, synthetic construct
  REGION 1..15: note = linker 15_aa
GGGGSGGGGSGGGGS

SEQ ID NO: 42 - protein, 25 aa, synthetic construct
  REGION 1..25: note = linker 25_aa
SSADDAKKDAAKKDDAKKDDAKKDG

SEQ ID NO: 43 - DNA, 45 bp, synthetic construct
  misc_feature 1..45: note = linker 15_base
  source 1..45: mol_type = other DNA
ggcggcggagggtcaggcggtggcgggtctggcggtggaggatcc

SEQ ID NO: 44 - DNA, 75 bp, synthetic construct
  misc_feature 1..75: note = linker 25_base
  source 1..75: mol_type = other DNA
agcagcgccgatgacgctaaaaaggacgccgccaaaaaggacgacgctaagaaagacgacgccaagaaggatgga

SEQ ID NO: 45 - DNA, 63 bp, synthetic construct
  misc_feature 1..63: note = Transmembrane regon
  source 1..63: mol_type = other DNA
atctacatctgggcgcccttggccgggacttgtggggtccttctcctgtcactggttatcacc

SEQ ID NO: 46 - DNA, 339 bp, Homo sapiens
  source 1..339: mol_type = genomic DNA
ctgagagtgaagttcagcaggagcgcagacgcccccgcgtaccagcagggccagaaccagctctataacgagctcaatctaggacgaagagaggagtacgatgttttggacaagagacgtggccgggaccctgagatggggggaaagccgagaaggaagaaccctcaggaaggcctgtacaatgaactgcagaaagataagatggcggaggcctacagtgagattgggatgaaaggcgagcgccggaggggcaaggggcacgatggcctttaccagggtctcagtacagccaccaaggacacctacgacgcccttcacatgcaggccctgccccctcgc

SEQ ID NO: 47 - DNA, 120 bp, Homo sapiens
  source 1..120: mol_type = genomic DNA
agtaagaggagcaggctcctgcacagtgactacatgaacatgactccccgccgccccgggcccacccgcaagcattaccagccctatgccccaccacgcgacttcgcagcctatcgctcc

SEQ ID NO: 48 - DNA, 138 bp, Homo sapiens
  source 1..138: mol_type = genomic DNA
cgtttctctgttgttaaacggggcagaaagaagctcctgtatatattcaaacaaccatttatgagaccagtacaaactactcaagaggaagatggctgtagctgccgatttccagaagaagaagaaggaggatgtgaa

SEQ ID NO: 49 - DNA, 531 bp, Homo sapiens
  source 1..531: mol_type = genomic DNA
atgttccatgtttcttttaggtatatctttggacttcctcccctgatccttgttctgttgccagtagcatcatctgattgtgatattgaaggtaaagatggcaaacaatatgagagtgttctaatggtcagcatcgatcaattattggacagcatgaaagaaattggtagcaattgcctgaataatgaatttaacttttttaaaagacatatctgtgatgctaataaggaaggtatgtttttattccgtgctgctcgcaagttgaggcaatttcttaaaatgaatagcactggtgattttgatctccacttattaaaagtttcagaaggcacaacaatactgttgaactgcactggccaggttaaaggaagaaaaccagctgccctgggtgaagcccaaccaacaaagagtttggaagaaaataaatctttaaaggaacagaaaaaactgaatgacttgtgtttcctaaagagactattacaagagataaaaacttgttggaataaaattttgatgggcactaaagaacac

SEQ ID NO: 50 - DNA, 294 bp, Homo sapiens
  source 1..294: mol_type = genomic DNA
atggccctgctactggccctcagcctgctggttctctggacttccccagccccaactctgagtggcaccaatgatgctgaagactgctgcctgtctgtgacccagaaacccatccctgggtacatcgtgaggaacttccactaccttctcatcaaggatggctgcagggtgcctgctgtagtgttcaccacactgaggggccgccagctctgtgcacccccagaccagccctgggtagaacgcatcatccagagactgcagaggacctcagccaagatgaagcgccgcagcagt

SEQ ID NO: 51 - protein, 116 aa, synthetic construct
  REGION 1..116: note = Clone: 2H9-1B5 VH region
QVTLKESGPGILQPSQTLSLTCSLSGFSLSTSGMGVSWIRQPSGKGLEWLAHIYWDDDTRYNPSLKRRLTISKDTSTNQVFLKITSVDTADTATYYCARNYGFDVWGAGTTVTVSS

SEQ ID NO: 52 - protein, 112 aa, synthetic construct
  REGION 1..112: note = Clone 2H9-1B5 VL region
DVVVTQTPLSLPVSLEDQASISCRSSRSLVHSNGKTYLQWYLQKPGQSPKLLIYSVSNRFSGVPDRFSGSGSGRDFTLKINRVEAEDLGVYFCSQSTHVPWTFGGGTKLEIK

SEQ ID NO: 53 - protein, 116 aa, synthetic construct
  REGION 1..116: note = Clone: 3C2-1B10 VH region
QVTLKESGPGILQPSQTLSLACSFSGFSLSTSGMGVSWIRQPSGKGLEWLAHIYWDDDRRYNPSLKSRLTISRDTSSNQVFLRITSVDTADTATYYCARNYGFDVWGAGTTVTVSS

SEQ ID NO: 54 - protein, 112 aa, synthetic construct
  REGION 1..112: note = Clone: 3C2-1B10 VL region
DVVVTQTPLSLPVSLGDQASISCRSSQSLVHSNGITYLQWYLQKPGQSPKLLIYKVSTRFSGVPDRFSGSGSGTDFTLRISRVEAEELGVYFCSQSTHIPWTFGGGTKLEIK